European Patent Application EP 4 141 117 A1, published March 1, 2023. Title: RNA NANOSTRUCTURES AND METHODS OF MAKING AND USING RNA NANOSTRUCTURES. Applicant: ARIZONA BOARD OF REGENTS ON BEHALF OF ARIZONA STATE UNIVERSITY. Application PCT/US2018/048973. The sequence listing filed with the application follows.

SEQUENCE LISTING (20 sequences)

SEQ ID NO: 1 - RNA, 2002 nt, Artificial Sequence
  source: /note="Description of Artificial Sequence: Synthetic polynucleotide"
gggagagagcucgagcgaacacuagccacuugaucacgcugagcgcucguacaaugaaacacaggugugucagugcuaugcacguucgaagagcuguaucagcguucgugugaaugaguucaacggaguguugacuaagccgguugcuacauuucuguagcacacauagucaagauuugcaccagacgauacucucccucaguccuguuuaugcaagucgucguaguccugacguacuuccuaagcucgucacuguacugaugauuccacugaucaagaugcacguaucuucaguuuccugaagaucggaguaggcacuauaaucgacaaguaacgcuuacgauuccaucacgagugacuuaccugaaccauaacugacaagggaccacgcagaggucauacucacaggacuucaaaucuugagucggguucgaucauuucugaucgagacaccagugugagguaaucguacgucacuugauaggagcucuaaguagaguugagagccuguuaacuagacacgaguaacgagguuagccuguacgagauaucgggcuauagugcggacacgauugcaccauuucuggugcaacgaaggugagcauguauggacaggucagugugacucaagucgauaguccaaguagguuaucgacucgcauagcucaaugacugucaucgccagaguaucuaggugucuaccucacgaaucgcgucguuacauuucuguaacgcucauaccgugcugaucuaugggacacgucgcuuauucuugggucaugacaguugccacaaacaaggcacgaccucacaccugcgaacuucaagcguuaggcugacguuacaugcuugcgugcacugauucguuuccgaaucagagaccuacgaagccagaguucguucacuaucauaagugcacugaugcauuugugccaacauugaaggcaucgagauaaacagccgucuuaaucaagugagcaccugagaucagcaugauucgucuauuucuagacgaaucaacuuccauucaggugccuugcuacuuaagacgggauuaacucucgaugcaacgugcauuggcacaacucgugaugugcacuuucacacuggaacgaacucuggcuucguaggucuguuugucauuucugacaaacugcacgcacuguuaguacgucagccacuuaaccgaaguucgucauaaguaggucgugcgacuacgauggcaacuucuacuuaccaagaauaagcgacgugucccauaauggaagucgguaugagguaugacuuucgucauacacgcgauuccacaaugugacaccuaacguuugaggcgaugaccugauacaagcuaugcaugguucaaaccuacuuggacuaucgacuugagaugauaguaccuguccaacuaacagcaccuucgauaccucguuuccgagguauucguguccugugucaggcccgauauuaauguguggcuaacccuuaggaacgugucuaguuaacaggcucucaacgucaugacgagcuccuaguagcaagcguacgauacauugugacuggugucuacuggauuucuccaguaacccgacuccgacuacaaaguccugacucauucaccucugcguggucccuugucaguugagucgaugguaagucaaugcaucaggaaucgugguuaagucuugucgaucugacacacuacuccgcuguccuguuuccaggacagacgugcauuagcaguuguggaaucaucaguacagugacgagucguuacuguacgucagcuuguuugcgacuugcaguuaaucgacugagggucaaacgugucugguguguagucggacuaugugacguucauuucugaacguaccggcuuagucaacacuccguugaugaguaugacacgaacgagucauuggcucuucgcuucaauguagcacugaacuuaugauguuucauacacauuacgcucagcgaacugcuauggcuaguguucggaucc

SEQ ID NO: 2 - DNA, 2002 bp, Artificial Sequence
  source: /note="Description of Artificial Sequence: Synthetic polynucleotide"
gggagagagctcgagcgaacactagccacttgatcacgctgagcgctcgtacaatgaaacacaggtgtgtcagtgctatgcacgttcgaagagctgtatcagcgttcgtgtgaatgagttcaacggagtgttgactaagccggttgctacatttctgtagcacacatagtcaagatttgcaccagacgatactctccctcagtcctgtttatgcaagtcgtcgtagtcctgacgtacttcctaagctcgtcactgtactgatgattccactgatcaagatgcacgtatcttcagtttcctgaagatcggagtaggcactataatcgacaagtaacgcttacgattccatcacgagtgacttacctgaaccataactgacaagggaccacgcagaggtcatactcacaggacttcaaatcttgagtcgggttcgatcatttctgatcgagacaccagtgtgaggtaatcgtacgtcacttgataggagctctaagtagagttgagagcctgttaactagacacgagtaacgaggttagcctgtacgagatatcgggctatagtgcggacacgattgcaccatttctggtgcaacgaaggtgagcatgtatggacaggtcagtgtgactcaagtcgatagtccaagtaggttatcgactcgcatagctcaatgactgtcatcgccagagtatctaggtgtctacctcacgaatcgcgtcgttacatttctgtaacgctcataccgtgctgatctatgggacacgtcgcttattcttgggtcatgacagttgccacaaacaaggcacgacctcacacctgcgaacttcaagcgttaggctgacgttacatgcttgcgtgcactgattcgtttccgaatcagagacctacgaagccagagttcgttcactatcataagtgcactgatgcatttgtgccaacattgaaggcatcgagataaacagccgtcttaatcaagtgagcacctgagatcagcatgattcgtctatttctagacgaatcaacttccattcaggtgccttgctacttaagacgggattaactctcgatgcaacgtgcattggcacaactcgtgatgtgcactttcacactggaacgaactctggcttcgtaggtctgtttgtcatttctgacaaactgcacgcactgttagtacgtcagccacttaaccgaagttcgtcataagtaggtcgtgcgactacgatggcaacttctacttaccaagaataagcgacgtgtcccataatggaagtcggtatgaggtatgactttcgtcatacacgcgattccacaatgtgacacctaacgtttgaggcgatgacctgatacaagctatgcatggttcaaacctacttggactatcgacttgagatgatagtacctgtccaactaacagcaccttcgatacctcgtttccgaggtattcgtgtcctgtgtcaggcccgatattaatgtgtggctaacccttaggaacgtgtctagttaacaggctctcaacgtcatgacgagctcctagtagcaagcgtacgatacattgtgactggtgtctactggatttctccagtaacccgactccgactacaaagtcctgactcattcacctctgcgtggtcccttgtcagttgagtcgatggtaagtcaatgcatcaggaatcgtggttaagtcttgtcgatctgacacactactccgctgtcctgtttccaggacagacgtgcattagcagttgtggaatcatcagtacagtgacgagtcgttactgtacgtcagcttgtttgcgacttgcagttaatcgactgagggtcaaacgtgtctggtgtgtagtcggactatgtgacgttcatttctgaacgtaccggcttagtcaacactccgttgatgagtatgacacgaacgagtcattggctcttcgcttcaatgtagcactgaacttatgatgtttcatacacattacgctcagcgaactgctatggctagtgttcggatcc

SEQ ID NO: 3 - RNA, 2035 nt, Artificial Sequence
  source: /note="Description of Artificial Sequence: Synthetic polynucleotide"
gggagaggauccgaacacuagccauagcaguucgcugagcguaauguguaugaaacaucauaaguucagugcuacauugaagcgaagagccaaugacucguucgugucauacucaucaacggaguguugacuaagccgguacguucagggagggugaacgucacauaguccgacuacacaccagacacguuugacccucagucgauuaacugcaagucgcaaacaagcugacguacaguaacgacucgucacuguacugaugauuccacaacugcuaaugcacgucuguccuggggagggcaggacagcggaguagugugucagaucgacaagacuuaaccacgauuccugaugcauugacuuaccaucgacucaacugacaagggaccacgcagaggugaaugagucaggacuuuguagucggagucggguuacuggagggaggguccaguagacaccagucacaauguaucguacgcuugcuacuaggagcucgucaugacguugagagccuguuaacuagacacguuccuaaggguuagccacacauuaauaucgggccugacacaggacacgaauaccucggggagggcgagguaucgaaggugcuguuaguuggacagguacuaucaucucaagucgauaguccaaguagguuugaaccaugcauagcuuguaucaggucaucgccucaaacguuaggugucacauuguggaaucgcguguaugacgggaggggucauaccucauaccgacuuccauuaugggacacgucgcuuauucuugguaaguagaaguugccaucguagucgcacgaccuacuuaugacgaacuucgguuaaguggcugacguacuaacagugcgugcaguuugucagggagggugacaaacagaccuacgaagccagaguucguuccagugugaaagugcacaucacgaguugugccaaugcacguugcaucgagaguuaaucccgucuuaaguagcaaggcaccugaauggaaguugauucgucuagaaauagacgaaucaugcugaucucaggugcucacuugauuaagacggcuguuuaucucgaugccuucaauguuggcacaaaugcaucagugcacuuaugauagugaacgaacucuggcuucguaggucucugauucggggagggcgaaucagugcacgcaagcauguaacgucagccuaacgcuugaaguucgcaggugugaggucgugccuuguuuguggcaacugucaugacccaagaauaagcgacgugucccauagaucagcacgguaugagcguuacagggaggguguaacgacgcgauucgugagguagacaccuagauacucuggcgaugacagucauugagcuaugcgagucgauaaccuacuuggacuaucgacuugagucacacugaccuguccauacaugcucaccuucguugcaccagggaggguggugcaaucguguccgcacuauagcccgauaucucguacaggcuaaccucguuacucgugucuaguuaacaggcucucaacucuacuuagagcuccuaucaagugacguacgauuaccucacacuggugucucgaucagggagggugaucgaacccgacucaagauuugaaguccugugaguaugaccucugcguggucccuugucaguuaugguucagguaagucacucgugauggaaucguaagcguuacuugucgauuauagugccuacuccgaucuucaggggagggcugaagauacgugcaucuugaucaguggaaucaucaguacagugacgagcuuaggaaguacgucaggacuacgacgacuugcauaaacaggacugagggagaguaucgucuggugcaaaucuugacuaugugugcuacagggaggguguagcaaccggcuuagucaacacuccguugaacucauucacacgaacgcugauacagcucuucgaacgugcauagcacugacacaccuguguuucauuguacgagcgcucagcgugaucaaguggcuaguguucgcucgag

SEQ ID NO: 4 - RNA, 2038 nt, Artificial Sequence
  source: /note="Description of Artificial Sequence: Synthetic polynucleotide"
gggagagagcucgagcgaacacuagccacuugaucacgcugagcgcucguacaaugaaacacaggugugucagugcuaugcacguucgaagagcuguaucagcguucgugugaaugaguucaacggaguguugacuaagccgguugcuacacccucccuguagcacacauagucaagauuugcaccagacgauacucucccucaguccuguuuaugcaagucgucguaguccugacguacuuccuaagcucgucacuguacugaugauuccacugaucaagaugcacguaucuucagcccuccccugaagaucggaguaggcacuauaaucgacaaguaacgcuuacgauuccaucacgagugacuuaccugaaccauaacugacaagggaccacgcagaggucauacucacaggacuucaaaucuugagucggguucgaucacccucccugaucgagacaccagugugagguaaucguacgucacuugauaggagcucuaaguagaguugagagccuguuaacuagacacgaguaacgagguuagccuguacgagauaucgggcuauagugcggacacgauugcaccacccucccuggugcaacgaaggugagcauguauggacaggucagugugacucaagucgauaguccaaguagguuaucgacucgcauagcucaaugacugucaucgccagaguaucuaggugucuaccucacgaaucgcgucguuacacccucccuguaacgcucauaccgugcugaucuaugggacacgucgcuuauucuugggucaugacaguugccacaaacaaggcacgaccucacaccugcgaacuucaagcguuaggcugacguuacaugcuugcgugcacugauucgcccuccccgaaucagagaccuacgaagccagaguucguucacuaucauaagugcacugaugcauuugugccaacauugaaggcaucgagauaaacagccgucuuaaucaagugagcaccugagaucagcaugauucgucuauuucuagacgaaucaacuuccauucaggugccuugcuacuuaagacgggauuaacucucgaugcaacgugcauuggcacaacucgugaugugcacuuucacacuggaacgaacucuggcuucguaggucuguuugucacccucccugacaaacugcacgcacuguuaguacgucagccacuuaaccgaaguucgucauaaguaggucgugcgacuacgauggcaacuucuacuuaccaagaauaagcgacgugucccauaauggaagucgguaugagguaugaccccucccgucauacacgcgauuccacaaugugacaccuaacguuugaggcgaugaccugauacaagcuaugcaugguucaaaccuacuuggacuaucgacuugagaugauaguaccuguccaacuaacagcaccuucgauaccucgcccuccccgagguauucguguccugugucaggcccgauauuaauguguggcuaacccuuaggaacgugucuaguuaacaggcucucaacgucaugacgagcuccuaguagcaagcguacgauacauugugacuggugucuacuggacccucccuccaguaacccgacuccgacuacaaaguccugacucauucaccucugcguggucccuugucaguugagucgaugguaagucaaugcaucaggaaucgugguuaagucuugucgaucugacacacuacuccgcuguccugcccuccccaggacagacgugcauuagcaguuguggaaucaucaguacagugacgagucguuacuguacgucagcuuguuugcgacuugcaguuaaucgacugagggucaaacgugucugguguguagucggacuaugugacguucacccucccugaacguaccggcuuagucaacacuccguugaugaguaugacacgaacgagucauuggcucuucgcuucaauguagcacugaacuuaugauguuucauacacauuacgcucagcgaacugcuauggcuaguguucggaucc

SEQ ID NO: 5 - RNA, 2035 nt, Artificial Sequence
  source: /note="Description of Artificial Sequence: Synthetic polynucleotide"
gggagaggauccgaacacuagccauagcaguucgcugagcguaauguguaugaaacaucauaaguucagugcuacauugaagcgaagagccaaugacucguucgugucauacucaucaacggaguguugacuaagccgguacguucaaaagaaaugaacgucacauaguccgacuacacaccagacacguuugacccucagucgauuaacugcaagucgcaaacaagcugacguacaguaacgacucgucacuguacugaugauuccacaacugcuaaugcacgucuguccugaaagaaacaggacagcggaguagugugucagaucgacaagacuuaaccacgauuccugaugcauugacuuaccaucgacucaacugacaagggaccacgcagaggugaaugagucaggacuuuguagucggagucggguuacuggaaaagaaauccaguagacaccagucacaauguaucguacgcuugcuacuaggagcucgucaugacguugagagccuguuaacuagacacguuccuaaggguuagccacacauuaauaucgggccugacacaggacacgaauaccucgaaagaaacgagguaucgaaggugcuguuaguuggacagguacuaucaucucaagucgauaguccaaguagguuugaaccaugcauagcuuguaucaggucaucgccucaaacguuaggugucacauuguggaaucgcguguaugacaaagaaagucauaccucauaccgacuuccauuaugggacacgucgcuuauucuugguaaguagaaguugccaucguagucgcacgaccuacuuaugacgaacuucgguuaaguggcugacguacuaacagugcgugcaguuugucaaaagaaaugacaaacagaccuacgaagccagaguucguuccagugugaaagugcacaucacgaguugugccaaugcacguugcaucgagaguuaaucccgucuuaaguagcaaggcaccugaauggaaguugauucgucuagaaauagacgaaucaugcugaucucaggugcucacuugauuaagacggcuguuuaucucgaugccuucaauguuggcacaaaugcaucagugcacuuaugauagugaacgaacucuggcuucguaggucucugauucgaaagaaacgaaucagugcacgcaagcauguaacgucagccuaacgcuugaaguucgcaggugugaggucgugccuuguuuguggcaacugucaugacccaagaauaagcgacgugucccauagaucagcacgguaugagcguuacaaaagaaauguaacgacgcgauucgugagguagacaccuagauacucuggcgaugacagucauugagcuaugcgagucgauaaccuacuuggacuaucgacuugagucacacugaccuguccauacaugcucaccuucguugcaccaaaagaaauggugcaaucguguccgcacuauagcccgauaucucguacaggcuaaccucguuacucgugucuaguuaacaggcucucaacucuacuuagagcuccuaucaagugacguacgauuaccucacacuggugucucgaucaaaagaaaugaucgaacccgacucaagauuugaaguccugugaguaugaccucugcguggucccuugucaguuaugguucagguaagucacucgugauggaaucguaagcguuacuugucgauuauagugccuacuccgaucuucagaaagaaacugaagauacgugcaucuugaucaguggaaucaucaguacagugacgagcuuaggaaguacgucaggacuacgacgacuugcauaaacaggacugagggagaguaucgucuggugcaaaucuugacuaugugugcuacaaaagaaauguagcaaccggcuuagucaacacuccguugaacucauucacacgaacgcugauacagcucuucgaacgugcauagcacugacacaccuguguuucauuguacgagcgcucagcgugaucaaguggcuaguguucgcucgag

SEQ ID NO: 6 - RNA, 2038 nt, Artificial Sequence
  source: /note="Description of Artificial Sequence: Synthetic polynucleotide"
gggagagagcucgagcgaacacuagccacuugaucacgcugagcgcucguacaaugaaacacaggugugucagugcuaugcacguucgaagagcuguaucagcguucgugugaaugaguucaacggaguguugacuaagccgguugcuacauuucuuuuguagcacacauagucaagauuugcaccagacgauacucucccucaguccuguuuaugcaagucgucguaguccugacguacuuccuaagcucgucacuguacugaugauuccacugaucaagaugcacguaucuucaguuucuuucugaagaucggaguaggcacuauaaucgacaaguaacgcuuacgauuccaucacgagugacuuaccugaaccauaacugacaagggaccacgcagaggucauacucacaggacuucaaaucuugagucggguucgaucauuucuuuugaucgagacaccagugugagguaaucguacgucacuugauaggagcucuaaguagaguugagagccuguuaacuagacacgaguaacgagguuagccuguacgagauaucgggcuauagugcggacacgauugcaccauuucuuuuggugcaacgaaggugagcauguauggacaggucagugugacucaagucgauaguccaaguagguuaucgacucgcauagcucaaugacugucaucgccagaguaucuaggugucuaccucacgaaucgcgucguuacauuucuuuuguaacgcucauaccgugcugaucuaugggacacgucgcuuauucuugggucaugacaguugccacaaacaaggcacgaccucacaccugcgaacuucaagcguuaggcugacguuacaugcuugcgugcacugauucguuucuuucgaaucagagaccuacgaagccagaguucguucacuaucauaagugcacugaugcauuugugccaacauugaaggcaucgagauaaacagccgucuuaaucaagugagcaccugagaucagcaugauucgucuauuucuagacgaaucaacuuccauucaggugccuugcuacuuaagacgggauuaacucucgaugcaacgugcauuggcacaacucgugaugugcacuuucacacuggaacgaacucuggcuucguaggucuguuugucauuucuuuugacaaacugcacgcacuguuaguacgucagccacuuaaccgaaguucgucauaaguaggucgugcgacuacgauggcaacuucuacuuaccaagaauaagcgacgugucccauaauggaagucgguaugagguaugacuuucuuugucauacacgcgauuccacaaugugacaccuaacguuugaggcgaugaccugauacaagcuaugcaugguucaaaccuacuuggacuaucgacuugagaugauaguaccuguccaacuaacagcaccuucgauaccucguuucuuucgagguauucguguccugugucaggcccgauauuaauguguggcuaacccuuaggaacgugucuaguuaacaggcucucaacgucaugacgagcuccuaguagcaagcguacgauacauugugacuggugucuacuggauuucuuuuccaguaacccgacuccgacuacaaaguccugacucauucaccucugcguggucccuugucaguugagucgaugguaagucaaugcaucaggaaucgugguuaagucuugucgaucugacacacuacuccgcuguccuguuucuuucaggacagacgugcauuagcaguuguggaaucaucaguacagugacgagucguuacuguacgucagcuuguuugcgacuugcaguuaaucgacugagggucaaacgugucugguguguagucggacuaugugacguucauuucuuuugaacguaccggcuuagucaacacuccguugaugaguaugacacgaacgagucauuggcucuucgcuucaauguagcacugaacuuaugauguuucauacacauuacgcucagcgaacugcuauggcuaguguucggaucc

SEQ ID NO: 7 - RNA, 2310 nt, Artificial Sequence
  source: /note="Description of Artificial Sequence: Synthetic polynucleotide"
gggagagagcucgagcgaacacuagccacuugaucacucgugcuucucguacauggaagcccagguguggagauaaggucuuagguuuuccuaagaugagcguuuaacgugcaucuugacucugauacaauuccauagacucauucaugucgcauaccucuguuuucagagguaaccacggguguagucgacugcguagucaaacgucgaucuacagcuaaucgaggcuuucuccaucguuuucgauggaaugauucggcaaacuaggacacgagaguaacgaaggaauguacaaucgacucgacauucaaccagcuuuugcugguuggaucgucgugugucaggcguuguccacuuaaccaguagacccuaaacagucacugacgacuaugcuuuugcauaguuaugguacaaugcaucauguacgaggagucgaugccauauagugaguaugcacgugagagacgaacuuuuguucgucuugacuuacuaccucacuaugcuagaucaagugaucgggauuucauaaguguuaagggcaucgcuauuuuuagcgaucgcaaguggugcugaucacgaccauauagaagucauggaaacugaucaaguagaugguguggcuuguuuucaagccacuugcguaugucaugacaaagccuuaguagcaagaugggacuugcacguucucauuggcgcauagguuuuccuaugcuucaggaguuacaugcuguaccucaaugguucauccaugccgcgacuacagcagcaacaaugaucguuuucgaucauucauagggucagugugacgugaaucguaacgcuuaugaaccacuaguuugcaggguuguauaugcguuuucgcauaucacuccacuggccuaauucgauaccuuccuaagcuccgcgaccugacacaguuagcucugucgaacuuuuguucgacaaggcacuuacuaucauguucgauacagaguaucugacugugugaugcauaagcaauggccacagcuuuugcuguggaccagcaguacuaacagcuuaagagagucauuguguuaugucgugagguacagcucacgucagaucuuuugaucugacuggucgaaucuacguacugguucaauaaugugucguaaucggaucagcaugauucgucuauuucuagacgaaucaacuuccaucgauuacguguacgaguugaaccaggucaugacuucgaccaaccaccuguuuucagguggugugagcugacauuguggacauaacauguaucagcucuuaagagcauguaacugcugguaacgacguuuucgucguuccauugcuucucgugaucacagucaacguuugaguaucgaacucacacugaagugccucugguauguuuucauaccaggagcuaacgcacuauagucgcggagucguuacugguaucgaauuaggccaguggagugcuuuagcuuuugcuaaagacaacccugucguagucugguucaugguuaagucgauucacgaugauaguacccuauggaucuuacuuuuguaagaucguugcugcacaaucuucggcauggaaucgacucugagguaccuguuaguacuccugaaaugucacuuuugugacaugccaaugagguucaaugagucccauucacuugauaaggcuuuuacguagaauacgcaacuacuaacuuuuguuaguagaccaucuauagcaguuguuuccaugacuucuauauggucguauggaaguccacuugcgugaacgauuuuucguucagcccuuaaccacaccugaaucccgacuugcuacucuagcauacacaauguguaagucaggcucugguuuuccagagcccucacguggaaugagucuauauggcugaaccaucucguacaaucacgaguguaccauaguaugaguuuucucauaccgucagugagauuagcuggucuacuaagcguuaggacaacgcuauagugccgacgaucucuagucguuuucgacuagaaaugucgagucgauuguacauuccucuuaggaacucgugucgacuacgaccgaaucauaguaaccuuuugguuacugaaagccuccuguuuagguagaucggauacucucuacgcaguaagauugucccgugguagauccucuuuugaggaucuugcgacaucauacucacuauggaaucaaugacuagucaagacauugaacaaacgcucaagucaucuuuugaugacuccuuaucucacuuaugaggcuuccaacacauuaaagcacgagaacugcuauggcuaguguucggaucc

SEQ ID NO: 8 - RNA, 2088 nt, Artificial Sequence
  source: /note="Description of Artificial Sequence: Synthetic polynucleotide"
gggagagagcucgagcgaacacuagccacuugaucaacuggacauacauuguguucaugccuguagucgaucugaauggcacuauauccauaaacacacgucgcugcguaggacuacgacgaaaaugagaguauccacagcauacauacucagauaguggucauaagucugcugugcaucgagaacagaagaaguagcaaggagcucaucacagucguuuucgacugugcaguuguagauuagcuaccgguugaugaaaccauuaaugaagcccacccggacugauuuccuaagaacucuugugauacucuccuugguuagucauugcgggagugaacacauuagugaacaugaagccauaaugcgaugacuuccauggagcaaacacaauguagaaacucaaugguucagccggauucuaagucguuuucgacuuaggauaguagggagauggacgauucggacuuaaccuagcuuguacaaucuuaucuaggcacauugaacuagaaggguaauguguggaccuuucuacuuugucaauauccgucaugacucagggacugaaugagugcugaucgcagugugaccauccccggguuucauagccuggggaaaacaagcccuuacaguagcacuuuugugcuaccguucgguccuguuuaguuugcagaacuaacagugccaaaguacuuaugacucccuugauauagacuaugcuuaggucaugacaggagcugcugauacaggaaccaaucucgugaugaguaaccuauagugcaacuacuucauacgcauguaacaaagguuaagugccgacuucaagucgaugugccgacaguaacacuuuuguguuacucauacuuguagcaguuucacagaaucuacacauacucuggaauggaagugcguguguuugcacguugcugauugaucacgagacaagggaacuaguuugucaauuucacaagcaccuacgacgucuuaggaaguaagucgacuaucaucccuuguuccuguuaguaagcacugucaagugauacugcucuauuucuagagcaguacuugcuaccagugcuuuacaugcugaacaagggucacacugcgacuuacaguaacgaacgucguaggugcuugugaaauugaucguagucuucccuuguaugcaucacaaucagcguucaaugaacacacgcugcugaucuccagaguauguguagauucugugaugaucaagcaaguaugcugcguaguuuucuacgcaggucggcacugaaccaugaagucggcuaacgcuuuuuguuacaugcguaugaaguaguuugugucaggguuacucugaugcauauugguucccaaugacucagcuccuucuacguacuaagcauagucuauaucaagggagcaggugugacuuuggcaagcauguaucugcaaaagcuaaucgaccgaacgucggucguuuucgaccgauguaagggcuuguuuuccccaggcuccguaugacggggauggaugauagucgaucagcugaguaugagucccugauacguagaggauauugacaaaguagaaagguccuguacgagcccuucuaaacgugcaugccuagaucgacuacaacaagcuaaagcguuaccgaaucguccaucucccuacuaucgucacaacuuuuguugugacaauccggcaucgacuuugaguuucuuaccucacuuugcuccgaucagcacaucgcauuauggcuucauguucaccucguacaucacucccguguaucagaaccaaggucaaacguacaagaguuucguuacuaucaguccgggugggcuucauuaauucauacggcaaccggucuaaacaguacaacugcguuacccuuuuggguaacgaugagcucucacuugauucuucuguucucgaugcacagcagcacaccugccacuaucacucauucuaugcugugacguuugacauuuucgcaaacuagcuacgcagcgacguguguuuauggacugacacacauucagauaagauuguggcaugaagugagguaauguccaguaacugcuauggcuaguguucggaucc

SEQ ID NO: 9 - RNA, 1838 nt, Artificial Sequence
  source: /note="Description of Artificial Sequence: Synthetic polynucleotide"
gggagaggauccgaacacuagccauagcaguucgcugagcguaauguguaugaaacaucauaaguucagugcuacauugaagcgaagagccaaugacucguucgugucauacucaucaacggaguguugacuaagccgaaaaaacauaguccgacuacacaccagacacguuugacccucagucgauuaacugcaagucgcaaacaagcugacguacaguaacgacucgucacuguacugaugauuccacaacugcuaaugcacgaaaaaaggaguagugugucagaucgacaagacuuaaccacgauuccugaugcauugacuuaccaucgacucaacugacaagggaccacgcagaggugaaugagucaggacuuuguagucggagucggaaaaaacaccagucacaauguaucguacgcuugcuacuaggagcucgucaugacguugagagccuguuaacuagacacguuccuaaggguuagccacacauuaauaucgggccugacacaggacacgaaaaaagaaggugcuguuaguuggacagguacuaucaucucaagucgauaguccaaguagguuugaaccaugcauagcuuguaucaggucaucgccucaaacguuaggugucacauuguggaaucgcaaaaaacauaccgacuuccauuaugggacacgucgcuuauucuugguaaguagaaguugccaucguagucgcacgaccuacuuaugacgaacuucgguuaaguggcugacguacuaacagugcgugcaaaaaagaccuacgaagccagaguucguuccagugugaaagugcacaucacgaguugugccaaugcacguugcaucgagaguuaaucccgucuuaaguagcaaggcaccugaauggaaguugauucgucuagaaauagacgaaucaugcugaucucaggugcucacuugauuaagacggcuguuuaucucgaugccuucaauguuggcacaaaugcaucagugcacuuaugauagugaacgaacucuggcuucguaggucaaaaaagcacgcaagcauguaacgucagccuaacgcuugaaguucgcaggugugaggucgugccuuguuuguggcaacugucaugacccaagaauaagcgacgugucccauagaucagcacgguaugaaaaaagcgauucgugagguagacaccuagauacucuggcgaugacagucauugagcuaugcgagucgauaaccuacuuggacuaucgacuugagucacacugaccuguccauacaugcucaccuucaaaaaacguguccgcacuauagcccgauaucucguacaggcuaaccucguuacucgugucuaguuaacaggcucucaacucuacuuagagcuccuaucaagugacguacgauuaccucacacuggugaaaaaaccgacucaagauuugaaguccugugaguaugaccucugcguggucccuugucaguuaugguucagguaagucacucgugauggaaucguaagcguuacuugucgauuauagugccuacuccaaaaaacgugcaucuugaucaguggaaucaucaguacagugacgagcuuaggaaguacgucaggacuacgacgacuugcauaaacaggacugagggagaguaucgucuggugcaaaucuugacuaugaaaaaacggcuuagucaacacuccguugaacucauucacacgaacgcugauacagcucuucgaacgugcauagcacugacacaccuguguuucauuguacgagcgcucagcgugaucaaguggcuaguguucgcucgagcucucucccuuuagugaggguuaauuaagcu

SEQ ID NO: 10 - RNA, 1838 nt, Artificial Sequence
  source: /note="Description of Artificial Sequence: Synthetic polynucleotide"
gggagagagcucgagcgaacacuagccacuugaucacgcugagcgcucguacaaugaaacacaggugugucagugcuaugcacguucgaagagcuguaucagcguucgugugaaugaguucaacggaguguugacuaagccguuuuuucauagucaagauuugcaccagacgauacucucccucaguccuguuuaugcaagucgucguaguccugacguacuuccuaagcucgucacuguacugaugauuccacugaucaagaugcacguuuuuuggaguaggcacuauaaucgacaaguaacgcuuacgauuccaucacgagugacuuaccugaaccauaacugacaagggaccacgcagaggucauacucacaggacuucaaaucuugagucgguuuuuucaccagugugagguaaucguacgucacuugauaggagcucuaaguagaguugagagccuguuaacuagacacgaguaacgagguuagccuguacgagauaucgggcuauagugcggacacguuuuuugaaggugagcauguauggacaggucagugugacucaagucgauaguccaaguagguuaucgacucgcauagcucaaugacugucaucgccagaguaucuaggugucuaccucacgaaucgcuuuuuucauaccgugcugaucuaugggacacgucgcuuauucuugggucaugacaguugccacaaacaaggcacgaccucacaccugcgaacuucaagcguuaggcugacguuacaugcuugcgugcuuuuuugaccuacgaagccagaguucguucacuaucauaagugcacugaugcauuugugccaacauugaaggcaucgagauaaacagccgucuuaaucaagugagcaccugagaucagcaugauucgucuauuucuagacgaaucaacuuccauucaggugccuugcuacuuaagacgggauuaacucucgaugcaacgugcauuggcacaacucgugaugugcacuuucacacuggaacgaacucuggcuucguaggucuuuuuugcacgcacuguuaguacgucagccacuuaaccgaaguucgucauaaguaggucgugcgacuacgauggcaacuucuacuuaccaagaauaagcgacgugucccauaauggaagucgguauguuuuuugcgauuccacaaugugacaccuaacguuugaggcgaugaccugauacaagcuaugcaugguucaaaccuacuuggacuaucgacuugagaugauaguaccuguccaacuaacagcaccuucuuuuuucguguccugugucaggcccgauauuaauguguggcuaacccuuaggaacgugucuaguuaacaggcucucaacgucaugacgagcuccuaguagcaagcguacgauacauugugacugguguuuuuuccgacuccgacuacaaaguccugacucauucaccucugcguggucccuugucaguugagucgaugguaagucaaugcaucaggaaucgugguuaagucuugucgaucugacacacuacuccuuuuuucgugcauuagcaguuguggaaucaucaguacagugacgagucguuacuguacgucagcuuguuugcgacuugcaguuaaucgacugagggucaaacgugucugguguguagucggacuauguuuuuucggcuuagucaacacuccguugaugaguaugacacgaacgagucauuggcucuucgcuucaauguagcacugaacuuaugauguuucauacacauuacgcucagcgaacugcuauggcuaguguucggauccucucccuauagugagucguauuagaauu

SEQ ID NO: 11 - RNA, 2632 nt, Artificial Sequence
  source: /note="Description of Artificial Sequence: Synthetic polynucleotide"
gggagagagcucgagcgaacacuagacuugaucacuucguuuagcgaaaucgacucuggauaguacauugaacgugacuccucauaagugcuuugaaguaauguguaggcuauagaucagcacggucacuuaacauuaggcaacgcuacucaauguuuucauugagugcuacacugucaugacugugcaugacuugcuacaguuuguccugauacauacagaucccgacuacagugcgacagauuagcuugccuucauguuugccguuuucggcaaaccacacgcauugcagaugcgccacgacuuaggaagaaugcaugacuuaaccacaucagaugaugcaucccgauagacauacucaagacuaguuaccucacuagcaaccuggugcgauguucaaagcuacgucguuuucgacguagcauggcgcuacaugcuuaaagaauaacguuugaaggcggcauauagugcauauggccgaugaaaccgguggcuaaguugacuuuuucgagagaacaggguuuucccuguucguagugguacacucagguauaaaagagugcuaucucuaaucugauaacuggccacuggugguaucucgguuugaugacuacgacauuguucacuaucauaaugcuagccuguucacaccgacagucucaauguuuucauugagaguacgagugaacguccacuuaucugaugauaguuugaucucacuaacagcgauagccugugagguacaauauccuacguagauccucuuggugcugaucccaaagucuuaucgagaucucauaguuaaccaguuuucugguuaagagagcgaccucguacaaccuauacguagcaaggcgacugacgaaugagucgugguuaucaaacguaaguuaggccuaguuuggacauucauacaugaguuuucucauguagggcagugaguugauauguccaccuagauaccaaauccucucugacacaguuucauguaugcaucaacccuucgagucauugguuaucaccacuuaugauauaucccagucagucguucgaucgucugcguguuuucacgcagagaauugcgcugcacguucauguauuuguagucggaagauagcuaacgcuucacguggggguuucauauagugucguguagacucaggaucgacgugauguuuucaucacguguagguaagucaccauauuuuggaaauagcacuguguguuguacaggagaguccguaauuccuaagcacgucuucuguuuagguuuggagcgagucgauaccugcgaccgcuaugaucaaggucuccaucuauuucuagauggagacuagcaguuuagcggucgcagguugaaccaugcuccaaacagcuaaucaagacgugucguuacuuuacggacuagucaacucaacacacuccugauguuccaaaauauggugacuuaccuacccuauaucuuuugauauaggcgauccugcaguuauccgacacuauccguaugacccacguggguuaagugcuaucuucaagauuguaauacaugguucaauggcgcaauucgacauuacuuuuguaauguccgaucgaacgacugacugggauauacaggugugggugauaacuguaucagcgaaggguaucacgagacaugaaacgcacuauaagaggauugacaccuaagguggacauaucaacucacugcccgaugcaucuuuugaugcaucugaaugucucguagucgccuaacuugauacucuuaaccacgugaguauggucagucgcucacuugaguauagguacacauuagucgcucuccaaagcacuuuugugcuuugcuaugagaucucgauaagacuuuggauggaaguccaagaggagucaugacggauauugacauugugaggcuaucgagcauguagagaucaacagugugacagauaaguggacguucacucguacacaccaccuuuugguggugucugucggugugaacaggcuagcauuucacacuggaacaaugcaaacuagaucaaaccguaggugucccaguggcagucuacaagauuagagcaucaggacuuuuauaccugaguguaccacuacuugcuagcuuuugcuagcaaucucgaaaacuccuguauagccaccucauacggcggccauauugugucagugccgccuagaguaucuauucuuuacuguuagugcgccauggugacuucuuuugaagucaccuuugaacaucgcaccagguugcuacacaauguacuagucuacucauucucuaucgggcucgugauucugauguaagcguuacaugcauucaguaacgaucguggcgcaucugcaaugcguguggagucaucuuuugaugacucaugaaggcacuaaacagugucgcacacaaucuuggaucuguacaaugacugacaaacuucaagugaucaugcacaucuacguaaguguagcugcgcaccuuuuggugcgcaagcguugccuaauguuaagugaccgacuuccauuauagccuuguacgagcuucaaagccacaccugggagucacaacgugcauacuauccaaugguucauucgcuaaacgaagaacugcuaucuaguguucggaucc

SEQ ID NO: 12 - RNA, 1684 nt, Artificial Sequence
  source: /note="Description of Artificial Sequence: Synthetic polynucleotide"
gggagauuacucauaagggcuggcuugguucacuaggagcuaguuggguagcccgucaccagugcguacagcccguucauccgcuuugcgauugcucacacaacgcuucgaguuuacccguucugcgauugaucgaaagaucaggacaucgacgggugaacucgaguugggaagugagcgaucgcaagcgaucgaaacggaaaacucgcugcuuaccguaugaauaggagguaccuucugccgguagucguucguucaguaagcugagcucgaaagagcuguaguaguugaacggacgacuaacuuagaucguagagaccgaggcauacgguuccuugaaaaaggacgcaaugaccucgguuucuacggucuaaguaaaucaauaucaccacuacuaccuaugccacgaaaacccauugccgaggauccacaauggugcucacgcguuuauguagcauuuugagcgggaucgguugagagaaaucucauggaguuacgcucaagaugcuagcacacgccgagccuauagagauggauccugcuucgaaagaagcuccuacggucucuaugggcucggugugugccuagcucguagcucuaacuccaaucaugguggaaaaugaguaguccaucgcagaguauucggccugugagcguuguuacggauuugcugcagcggauggaguuuaugcgaaagcauagacucucgaucgcgcagcagauccguauucccaaccacaggucgaauaccgauguccggacugcucaaaaagagcgggguuagcaugcguugccaucucaacaucuccguacugcacucuacaugacaaguacgaggguaucuuguucgugagaucguucaugguagcacgcagcuucggcugaggagcgauccacaacgcucuagaaauagagcuggugacaucgcucuucagccgcuccuaggugcuaucaugaacccuuaugagaacaaaaagucgcgugggccccaaugccuagagcuaaaugcgaaaggugcaagcuacgcacagcgucugauaaggcgagugaaaacucgucuuaguucgucuugugcguggcuugccgcgauuccauuuaguucuaggucgucuaucccaugcgacaaaaagauauccucccucugaccauguagcgugcagugcggagaagaggugugagacgcgcaugcugcguugaaaaacgcucgaaaaccgucucauaccucucuccgugauaucaguaggauucgucagaggcgcaugaaaaugcgguacuugugaauccugcugauauuacggaguguugagguggcaaguuuucgaaaccucgcucccaccgugauaccgauccgagcuaugagcuagcauaaaugcgugaguaccauugccguaggacggcgauggguugccucagacgcagcccuaguuaucuaccuuucgauccuuggccacuucauuggggacuucgaaagaaguauagacgaaaguggcuaaggaugaaucgcgagauaauuagggcuagacgaacggcaaaaaacgugguauagcagcuuacggugauguugauuuccggcaggagguacuuccuauuucauugcgaagcggcgagaaaagcugugcgcacguugugggggcuacucaacuagaagcugcugaaccgagccagcgaucucacguaaucuccc

SEQ ID NO: 13 - RNA, 6337 nt, Artificial Sequence
  source: /note="Description of Artificial Sequence: Synthetic polynucleotide"
gggagaggauccaacauggagugcggauaugguucgcuaagggauucccugaaugcgaacucuaucaacugucgauaccuggagacgaugcugaucgaccugucaugggcgaaaaccuauaccgauguaaacuccguauauucauuuugcucuaguccaguccuggagguuacuucggaaaaaaguaccgcaguggugaagcguguccuccauacaccuccgcaagguauucacuuuugugaucauaguuauggguguaugaggauaugcacuucacuaugcagaugugagauagauguccgugggcagaugucagcgaaccgcgaagacucgcaaugaaaaaacgagugaagggcgucuuggcgcguccuugucucacccaacuggcuugugguuagagcuugacucugggauaugaccaucuuggucacuaauuuaggacugcccuaaccucccuaauggaugcgggugauaaguucugaaugucacguuugcaaauagcccuuaauguucccguacuguggcacgagcaaaaaaccuuacaccuaaggcgauacucacuucaacuguguguaucacauuaggugccuacgguaaacucaucgucuaguucugggacuguuucgucugguugaacguuauaauagacacgauaccugguucuaccauucgccgauccauuuggucuucgaaaaaacgagggagaaucacucuaucaaagaugcaccucguagcgagugaguggaacuucauaaagggaagucauggccggucagacuucuggcacugauaugcaacaucaguacagucuuaaguuccagccgaaagugcgguuggcaucucuuaggacacagagcgauuuuggacugguagcugaccgcaugaaaaaaggaacgacgugucgaaaggucccgguaguagcucccucauuccacuuggcuaaacguucaacacguaucgaguugguuuagguaguucgcagacgcacaaacgaaggcagguaaaacuuggcaaguugcgucguggcacgucauaccaguguugaaaaaacggcuauguagugucuagcugucaauacccguacccaucugaugguugcaggaugauuaggucgaaacgaagucucugaucugaggucgucugaagcuaaguaauaccuggcuaacuugacuaacucguacucauacucagcuuucucacauucugugcucaaaaucugcauugacugcaacgguccaaaaaagcgaccuucugugugaauaugaauacuaagcgggaguugaagaauagcucacagacagacacaaccuacaaaaugaaugagcaguccguguaagcucgcauugcucacuucagccuucgggcgcuauagccauuauuaugauccaacucgaucgaaaaaagguacuacguagauuuggccgacaccagauugcccguaccgacaaugcgguuucuuuguaaacugggcacuuacgaucauagggagcugguuacgaacggcauccgacaggaaucuagcucgaugcaugggauaguacuguccacauccagccgucccagagauagguagauugggaaaaaacgaucgguacugaucucuggugucugacaaacaccuccgcacucauuugagcaugagccaauguauaaguugcaccagaaucgcucugguaugucuaacaucugcaacaucuuaagggcagucaugacuacugaccguagucggcuagagcaccgugaggccaaaugauccuccagaaaaaagcacugaguugacaccauccgagaguauggagcacuagcuaucaugacgagguucccaguugaagucagaaucuugauggacgaagccuacuacuaccugcuguugguacauggauaagauuggcuuaguaggucauccaagacugggccuuggaaaaaaccacgguuugugaccaugaucgucccaugcauacugaaaucaucacuaguugcggaguacgagucgagcugugcagugcaaacuaaucccuuucggcggucacauaguccugaacgccguccuuaucaccgaaaucuuccaacaaagcauggcucguauaggugcccagucgacuacuggauacuggaaaaaacggacuuuagacagcacccucaaucuaugaucgguccagugguuaguucguuucugcgaguuuaccuugcaucaggauaugacaccucggguguugaagccugaauagagagccgguucgaucuugugucuacugaacgcaguguagcguuagcaaaaaagacacuauccugaagcacgcuauguucguaauucagccgacucgcauuauugcuggagcuucagcucggccuugacugagugcacucaggcauaucagucaacacagcaacuuccuacgacuguccuaaaucaacacugcuagucacgugugucuaucgucucgaccugcaagcaugggugucgucgaaaaaagcucacgcuguacaaccuucaccccauagugauagccacagaaaagccucugaacaccaaccagacggucgaaaagaaauguaagcucacugcgucuggugcguugacaagaagacccauuaugagcuuacgugcucucacguaggcacuauccaaaaaaggaguaaaggcgaacguucgcagcaguuuacucggugguuuaucucugaggucacgucgaccuaagucccaugaugacguccagacaaccuucccuugcuuccaaggcuuuggagguaugcuagagucaagaauuacucugcaucgagucaucaagcauucaguacuauuagauuggagcacgacacaaaaaagcaucuucaauuaggcuuaucugagacaucuggucaggucaccgaguaccagaugucgguagaaccaaagaugacauaacagugaucaaccgcaacuuacuguacccuacacgagauauguccgcuauagcgucaaacgcagguacugcgauggaaaaaacagcaguagcacaggcuuaacaucaaucugguggucaccucuauagggcuagagugacggguaucgguuaugacaguguugcagucagcaggugcauugucuucgucgagcaguaagcggauagacaagggucgacuuggucuauuaucauguaacacuccauuaccuggucuagaaauagaccagguaccacuacauuacaugaagucuucgcaagucgacaggcuauaauccgcuucaaauggaacgaagacacgacuuaagcugacuggguaugacucauaaccgugcuguugcacucuagguuggaucaggugaccaguuacgcuauguuaagccugugcuacugcugaaaaaaccaucgcgcauuguccguuugacaugcgauaggacauauccaaccaucgguacagucguaauacguugaucacccacucaccaucuuuguacagguagacaucuggacaagccagaccugacguaaacguucagauaaguagcgaacaagaugcaaaaaagugucgugcuccaaucuaauaguagaguagacuugaugaccaucuaucgaguaauucacagugaaagcauaccgugucuaucuuggaagcucaacucaguugucuguuaccugccaugggacuacuccauccgugaccugcugaaguaaccaccgauguugagucugcgaacguucgccuuuacuccaaaaaaggauaguuaugaucggagagcacaccauuguauaaugggugaucagagcaacgcacguacauaugugagcuuagucugaccuucgaccgcacucguuguguucagaaagaugguuguggcuaagcaaccagggugaaggacaguugacgugagcaaaaaacgacgacacccaugcuugcagguccacagacaagacacacuccucauacaguguugacgucacgaagucguagucccagaauguguugacaacggacucugagugccuaaaccaaaggccgaggaaauuggccagcaaucucauucaucggcugaagagacgguauagcgugcuucaggauagugucaaaaaagcuaacgauuccugucguucagugcucuuucgaucgaaccuagccaggauucaggccgugcuuaccgagguguagacuguagaugcaaguaucgcaggcagaaacguagggaggacuggaccuacgacucauugaggguugacagguaaguccgaaaaaaccaguauccaguagucgacugggcuauugcuggagccauggaauaccugaagauuuccauaucgcggacggcgccuaauguuaugugaccuuguaugaggauuagucaaguggacacagcucguuaucgcuuccgcaacgcuauucuauuucaguacucuuucaacgaucauggucacaaaccguggaaaaaaccaaggcauguggacggaugaccaucacuugcaaucuuauagaaagcucaacagcauccuuaucuaggcuucgagagaugcgauucugaucauuggagggaaccucacgugacaagcuagugagaugauuucucggauguacggaguucagugcaaaaaacuggaggaucauuuggccucacggccaagguaccgacuacucaccacugucaugacuagucaagggauguugcgccuuagggacauaccacuugguaccuggugcaucgacacgauuggcucacaugugacugagugcgcacacagaugucagacagucgucuacaguaccgaucgaaaaaacccaaucuaccuuagacgacgacggcuggccagucuuaguacuauugaaagagucgagcuagcuacacugcggaugccaccgucucccagcucccgccuacguuaagugccacucaacaaaagaaaccaguaccuggguacgggagcguaacugucggccaaaucuacguaguaccaaaaaacgaucgacccuauagauaauaauguaucgcaugcccgaagcagagauagagcaaugcacaaugguacggacugaaugcgaguuuuguagggaaagagcgucugugauagugaugucaacuccccaagugauuucauauugagguguuaggucgcaaaaaaggaccguugcagucaaugcagaugucacaugcagaaugugccauguacgaguaugaagcgauaauagucaaguggcucucuuauuacuuccaauuucacgaccucacuucuuguacuucguugauggaguaucauccugucguguagagaugggucaacagcaugacagcuagacacuacauagccgaaaaaacaacacucaacacuggugccacgaguauuacggccaaguugacgucaucuucguuugauauguaccgaacuacacucagucacucgauacuaagcacgcguuuagcuugcacugaugagggaggauaaggagggaccuuacuuauacucguuccaaaaaacaugcggucagcuaccaguccaaguaccaaguguguccuauccaucaacaaccgcaucauacaauggaacuuacauauccucugauguuaguccguugugccagaacauuucuuggccaugaugaguugauaugaaguuuguuauguucgcuacguuaagucgcuuugauagagugauucucccucgaaaaaacgaagacacugcucgucggcgaauuaccuguacagguaucuccaaagcuauaacguuaacgagugcgaaacaggaaguugccuagacgaucugcgauacguaggcauucaggacgauacacacuccaaugaugaguaucagauguuauguaaggaaaaaagcucgugccacaguacgggaacaccuugacuuauuugcaagucaugauuucagaacgcgauaugcgcauccauaacuaaccuuagggcaucgugacguuagugaccggcuuuuccauaucccuucacugugcucuaaccuacucgguguuggguguauagccuacgcgccaagacgcccuucacucgaaaaaacauugcguaauagaccgguucgcuacguuuaccccacggaucgaugcaucacaucugugguugcuagugcauagugacuagcacccauaagagucguaacaaaagucuuuguugugcggagguaaucaucugacacgcuggucaguagcgguacaaaaaaccgaaguaaccuccaggacuggauaccuuggaaaugaauagugucaacuuacaucgcagcaauauuucgcccagcugucuacgaucagcugucugugcagguaucguuguacaguagaguucgucuacucggaaucccuccuaauugcauauccguguaguggguuggauccucucgagcucucccuuuag

SEQ ID NO: 14 - DNA, 929 bp, Artificial Sequence
  source: /note="Description of Artificial Sequence: Synthetic polynucleotide"
gaattctaatacgactcactatagggagaggatccgaacactagccatagcagttcgctgagcgtaatgtgtatgaaacatcataagttcagtgctacattgaagcgaagagccaatgactcgttcgtgtcatactcatcaacggagtgttgactaagccgaaaaaacatagtccgactacacaccagacacgtttgaccctcagtcgattaactgcaagtcgcaaacaagctgacgtacagtaacgactcgtcactgtactgatgattccacaactgctaatgcacgaaaaaaggagtagtgtgtcagatcgacaagacttaaccacgattcctgatgcattgacttaccatcgactcaactgacaagggaccacgcagaggtgaatgagtcaggactttgtagtcggagtcggaaaaaacaccagtcacaatgtatcgtacgcttgctactaggagctcgtcatgacgttgagagcctgttaactagacacgttcctaagggttagccacacattaatatcgggcctgacacaggacacgaaaaaagaaggtgctgttagttggacaggtactatcatctcaagtcgatagtccaagtaggtttgaaccatgcatagcttgtatcaggtcatcgcctcaaacgttaggtgtcacattgtggaatcgcaaaaaacataccgacttccattatgggacacgtcgcttattcttggtaagtagaagttgccatcgtagtcgcacgacctacttatgacgaacttcggttaagtggctgacgtactaacagtgcgtgcaaaaaagacctacgaagccagagttcgttccagtgtgaaagtgcacatcacgagttgtgccaatgcacgttgcatcgagagttaatcccgtcttaagtagcaaggcacctgaatggaagttgattcgtctaga

SEQ ID NO: 15 - DNA, 939 bp, Artificial Sequence
  source: /note="Description of Artificial Sequence: Synthetic polynucleotide"
tctagaaatagacgaatcatgctgatctcaggtgctcacttgattaagacggctgtttatctcgatgccttcaatgttggcacaaatgcatcagtgcacttatgatagtgaacgaactctggcttcgtaggtcaaaaaagcacgcaagcatgtaacgtcagcctaacgcttgaagttcgcaggtgtgaggtcgtgccttgtttgtggcaactgtcatgacccaagaataagcgacgtgtcccatagatcagcacggtatgaaaaaagcgattcgtgaggtagacacctagatactctggcgatgacagtcattgagctatgcgagtcgataacctacttggactatcgacttgagtcacactgacctgtccatacatgctcaccttcaaaaaacgtgtccgcactatagcccgatatctcgtacaggctaacctcgttactcgtgtctagttaacaggctctcaactctacttagagctcctatcaagtgacgtacgattacctcacactggtgaaaaaaccgactcaagatttgaagtcctgtgagtatgacctctgcgtggtcccttgtcagttatggttcaggtaagtcactcgtgatggaatcgtaagcgttacttgtcgattatagtgcctactccaaaaaacgtgcatcttgatcagtggaatcatcagtacagtgacgagcttaggaagtacgtcaggactacgacgacttgcataaacaggactgagggagagtatcgtctggtgcaaatcttgactatgaaaaaacggcttagtcaacactccgttgaactcattcacacgaacgctgatacagctcttcgaacgtgcatagcactgacacacctgtgtttcattgtacgagcgctcagcgtgatcaagtggctagtgttcgctcgagctctctccctttagtgagggttaattaagctt

SEQ ID NO: 16 - DNA, 3185 bp, Artificial Sequence
  source: /note="Description of Artificial Sequence: Synthetic polynucleotide"
gaattctaatacgactcactatagggagaggatccaacatggagtgcggatatggttcgctaagggattccctgaatgcgaactctatcaactgtcgatacctggagacgatgctgatcgacctgtcatgggcgaaaacctataccgatgtaaactccgtatattcattttgctctagtccagtcctggaggttacttcggaaaaaagtaccgcagtggtgaagcgtgtcctccatacacctccgcaaggtattcacttttgtgatcatagttatgggtgtatgaggatatgcacttcactatgcagatgtgagatagatgtccgtgggcagatgtcagcgaaccgcgaagactcgcaatgaaaaaacgagtgaagggcgtcttggcgcgtccttgtctcacccaactggcttgtggttagagcttgactctgggatatgaccatcttggtcactaatttaggactgccctaacctccctaatggatgcgggtgataagttctgaatgtcacgtttgcaaatagcccttaatgttcccgtactgtggcacgagcaaaaaaccttacacctaaggcgatactcacttcaactgtgtgtatcacattaggtgcctacggtaaactcatcgtctagttctgggactgtttcgtctggttgaacgttataatagacacgatacctggttctaccattcgccgatccatttggtcttcgaaaaaacgagggagaatcactctatcaaagatgcacctcgtagcgagtgagtggaacttcataaagggaagtcatggccggtcagacttctggcactgatatgcaacatcagtacagtcttaagttccagccgaaagtgcggttggcatctcttaggacacagagcgattttggactggtagctgaccgcatgaaaaaaggaacgacgtgtcgaaaggtcccggtagtagctccctcattccacttggctaaacgttcaacacgtatcgagttggtttaggtagttcgcagacgcacaaacgaaggcaggtaaaacttggcaagttgcgtcgtggcacgtcataccagtgttgaaaaaacggctatgtagtgtctagctgtcaatacccgtacccatctgatggttgcaggatgattaggtcgaaacgaagtctctgatctgaggtcgtctgaagctaagtaatacctggctaacttgactaactcgtactcatactcagctttctcacattctgtgctcaaaatctgcattgactgcaacggtccaaaaaagcgaccttctgtgtgaatatgaatactaagcgggagttgaagaatagctcacagacagacacaacctacaaaatgaatgagcagtccgtgtaagctcgcattgctcacttcagccttcgggcgctatagccattattatgatccaactcgatcgaaaaaaggtactacgtagatttggccgacaccagattgcccgtaccgacaatgcggtttctttgtaaactgggcacttacgatcatagggagctggttacgaacggcatccgacaggaatctagctcgatgcatgggatagtactgtccacatccagccgtcccagagataggtagattgggaaaaaacgatcggtactgatctctggtgtctgacaaacacctccgcactcatttgagcatgagccaatgtataagttgcaccagaatcgctctggtatgtctaacatctgcaacatcttaagggcagtcatgactactgaccgtagtcggctagagcaccgtgaggccaaatgatcctccagaaaaaagcactgagttgacaccatccgagagtatggagcactagctatcatgacgaggttcccagttgaagtcagaatcttgatggacgaagcctactactacctgctgttggtacatggataagattggcttagtaggtcatccaagactgggccttggaaaaaaccacggtttgtgaccatgatcgtcccatgcatactgaaatcatcactagttgcggagtacgagtcgagctgtgcagtgcaaactaatccctttcggcggtcacatagtcctgaacgccgtccttatcaccgaaatcttccaacaaagcatggctcgtataggtgcccagtcgactactggatactggaaaaaacggactttagacagcaccctcaatctatgatcggtccagtggttagttcgtttctgcgagtttaccttgcatcaggatatgacacctcgggtgttgaagcctgaatagagagccggttcgatcttgtgtctactgaacgcagtgtagcgttagcaaaaaagacactatcctgaagcacgctatgttcgtaattcagccgactcgcattattgctggagcttcagctcggccttgactgagtgcactcaggcatatcagtcaacacagcaacttcctacgactgtcctaaatcaacactgctagtcacgtgtgtctatcgtctcgacctgcaagcatgggtgtcgtcgaaaaaagctcacgctgtacaaccttcaccccatagtgatagccacagaaaagcctctgaacaccaaccagacggtcgaaaagaaatgtaagctcactgcgtctggtgcgttgacaagaagacccattatgagcttacgtgctctcacgtaggcactatccaaaaaaggagtaaaggcgaacgttcgcagcagtttactcggtggtttatctctgaggtcacgtcgacctaagtcccatgatgacgtccagacaaccttcccttgcttccaaggctttggaggtatgctagagtcaagaattactctgcatcgagtcatcaagcattcagtactattagattggagcacgacacaaaaaagcatcttcaattaggcttatctgagacatctggtcaggtcaccgagtaccagatgtcggtagaaccaaagatgacataacagtgatcaaccgcaacttactgtaccctacacgagatatgtccgctatagcgtcaaacgcaggtactgcgatggaaaaaacagcagtagcacaggcttaacatcaatctggtggtcacctctatagggctagagtgacgggtatcggttatgacagtgttgcagtcagcaggtgcattgtcttcgtcgagcagtaagcggatagacaagggtcgacttggtctattatcatgtaacactccattacctggtctaga

SEQ ID NO: 17 - DNA, 3199 bp, Artificial Sequence
  source: /note="Description of Artificial Sequence: Synthetic polynucleotide"
tctagaaatagaccaggtaccactacattacatgaagtcttcgcaagtcgacaggctataatccgcttcaaatggaacgaagacacgacttaagctgactgggtatgactcataaccgtgctgttgcactctaggttggatcaggtgaccagttacgctatgttaagcctgtgctactgctgaaaaaaccatcgcgcattgtccgtttgacatgcgataggacatatccaaccatcggtacagtcgtaatacgttgatcacccactcaccatctttgtacaggtagacatctggacaagccagacctgacgtaaacgttcagataagtagcgaacaagatgcaaaaaagtgtcgtgctccaatctaatagtagagtagacttgatgaccatctatcgagtaattcacagtgaaagcataccgtgtctatcttggaagctcaactcagttgtctgttacctgccatgggactactccatccgtgacctgctgaagtaaccaccgatgttgagtctgcgaacgttcgcctttactccaaaaaaggatagttatgatcggagagcacaccattgtataatgggtgatcagagcaacgcacgtacatatgtgagcttagtctgaccttcgaccgcactcgttgtgttcagaaagatggttgtggctaagcaaccagggtgaaggacagttgacgtgagcaaaaaacgacgacacccatgcttgcaggtccacagacaagacacactcctcatacagtgttgacgtcacgaagtcgtagtcccagaatgtgttgacaacggactctgagtgcctaaaccaaaggccgaggaaattggccagcaatctcattcatcggctgaagagacggtatagcgtgcttcaggatagtgtcaaaaaagctaacgattcctgtcgttcagtgctctttcgatcgaacctagccaggattcaggccgtgcttaccgaggtgtagactgtagatgcaagtatcgcaggcagaaacgtagggaggactggacctacgactcattgagggttgacaggtaagtccgaaaaaaccagtatccagtagtcgactgggctattgctggagccatggaatacctgaagatttccatatcgcggacggcgcctaatgttatgtgaccttgtatgaggattagtcaagtggacacagctcgttatcgcttccgcaacgctattctatttcagtactctttcaacgatcatggtcacaaaccgtggaaaaaaccaaggcatgtggacggatgaccatcacttgcaatcttatagaaagctcaacagcatccttatctaggcttcgagagatgcgattctgatcattggagggaacctcacgtgacaagctagtgagatgatttctcggatgtacggagttcagtgcaaaaaactggaggatcatttggcctcacggccaaggtaccgactactcaccactgtcatgactagtcaagggatgttgcgccttagggacataccacttggtacctggtgcatcgacacgattggctcacatgtgactgagtgcgcacacagatgtcagacagtcgtctacagtaccgatcgaaaaaacccaatctaccttagacgacgacggctggccagtcttagtactattgaaagagtcgagctagctacactgcggatgccaccgtctcccagctcccgcctacgttaagtgccactcaacaaaagaaaccagtacctgggtacgggagcgtaactgtcggccaaatctacgtagtaccaaaaaacgatcgaccctatagataataatgtatcgcatgcccgaagcagagatagagcaatgcacaatggtacggactgaatgcgagttttgtagggaaagagcgtctgtgatagtgatgtcaactccccaagtgatttcatattgaggtgttaggtcgcaaaaaaggaccgttgcagtcaatgcagatgtcacatgcagaatgtgccatgtacgagtatgaagcgataatagtcaagtggctctcttattacttccaatttcacgacctcacttcttgtacttcgttgatggagtatcatcctgtcgtgtagagatgggtcaacagcatgacagctagacactacatagccgaaaaaacaacactcaacactggtgccacgagtattacggccaagttgacgtcatcttcgtttgatatgtaccgaactacactcagtcactcgatactaagcacgcgtttagcttgcactgatgagggaggataaggagggaccttacttatactcgttccaaaaaacatgcggtcagctaccagtccaagtaccaagtgtgtcctatccatcaacaaccgcatcatacaatggaacttacatatcctctgatgttagtccgttgtgccagaacatttcttggccatgatgagttgatatgaagtttgttatgttcgctacgttaagtcgctttgatagagtgattctccctcgaaaaaacgaagacactgctcgtcggcgaattacctgtacaggtatctccaaagctataacgttaacgagtgcgaaacaggaagttgcctagacgatctgcgatacgtaggcattcaggacgatacacactccaatgatgagtatcagatgttatgtaaggaaaaaagctcgtgccacagtacgggaacaccttgacttatttgcaagtcatgatttcagaacgcgatatgcgcatccataactaaccttagggcatcgtgacgttagtgaccggcttttccatatcccttcactgtgctctaacctactcggtgttgggtgtatagcctacgcgccaagacgcccttcactcgaaaaaacattgcgtaatagaccggttcgctacgtttaccccacggatcgatgcatcacatctgtggttgctagtgcatagtgactagcacccataagagtcgtaacaaaagtctttgttgtgcggaggtaatcatctgacacgctggtcagtagcggtacaaaaaaccgaagtaacctccaggactggataccttggaaatgaatagtgtcaacttacatcgcagcaatatttcgcccagctgtctacgatcagctgtctgtgcaggtatcgttgtacagtagagttcgtctactcggaatccctcctaattgcatatccgtgtagtgggttggatcctctcgagctctccctttagtgagggttaattaagctt

SEQ ID NO: 18 - protein, 28 aa, Artificial Sequence
  source: /note="Description of Artificial Sequence: Synthetic peptide"
CTKDNNLLGRFELSGGGSKKKKKKKKKK

SEQ ID NO: 19 - protein, 14 aa, Homo sapiens
TKDNNLLGRFELSG

SEQ ID NO: 20 - protein, 14 aa, Mus sp.
TRDNNLLGRFELSG